European Patent Application EP 4 356 933 A1, published April 24, 2024. Title: COMPOSITION FOR IN-VIVO DELIVERING mRNA CONTAINING MODIFIED NUCLEOTIDE. Applicant: EYEGENE INC. The sequence listing filed with the application follows.

SEQUENCE LISTING (4 sequences)

SEQ ID NO: 1 - RNA, 936 nt, synthetic construct
  source 1..936: mol_type = other RNA
atgaccagcaaggtgtacgaccccgagcagcggaagcggatgatcaccggcccccagtggtgggcccggtgcaagcagatgaacgtgctggacagcttcatcaactactacgacagcgagaagcacgccgagaacgccgtgatcttcctgcacggcaacgccgccagcagctacctgtggcggcacgtggtgccccacatcgagcccgtggcccggtgcatcatccccgacctgatcggcatgggcaagagcggcaagagcggcaacggcagctaccggctgctggaccactacaagtacctgaccgcctggttcgagctgctgaacctgcccaagaagatcatcttcgtgggccacgactggggcgcctgcctggccttccactacagctacgagcaccaggacaagatcaaggccatcgtgcacgccgagagcgtggtggacgtgatcgagagctgggacgagtggcccgacatcgaggaggacatcgccctgatcaagagcgaggagggcgagaagatggtgctggagaacaacttcttcgtggagaccatgctgcccagcaagatcatgcggaagctggagcccgaggagttcgccgcctacctggagcccttcaaggagaagggcgaggtgcggcggcccaccctgagctggccccgggagatccccctggtgaagggcggcaagcccgacgtggtgcagatcgtgcggaactacaacgcctacctgcgggccagcgacgacctgcccaagatgttcatcgagagcgaccccggcttcttcagcaacgccatcgtggagggcgccaagaagttccccaacaccgagttcgtgaaggtgaagggcctgcacttcagccaggaggacgcccccgacgagatgggcaagtacatcaagagcttcgtggagcgggtgctgaagaacgagcagtga

SEQ ID NO: 2 - protein, 311 aa, synthetic construct
MTSKVYDPEQRKRMITGPQWWARCKQMNVLDSFINYYDSEKHAENAVIFLHGNAASSYLWRHVVPHIEPVARCIIPDLIGMGKSGKSGNGSYRLLDHYKYLTAWFELLNLPKKIIFVGHDWGACLAFHYSYEHQDKIKAIVHAESVVDVIESWDEWPDIEEDIALIKSEEGEKMVLENNFFVETMLPSKIMRKLEPEEFAAYLEPFKEKGEVRRPTLSWPREIPLVKGGKPDVVQIVRNYNAYLRASDDLPKMFIESDPGFFSNAIVEGAKKFPNTEFVKVKGLHFSQEDAPDEMGKYIKSFVERVLKNEQ

SEQ ID NO: 3 - RNA, 3813 nt, synthetic construct
  source 1..3813: mol_type = other RNA
atgttcgtgttcctggtgctgctgcccctggtgagcagccagtgcgtgaacctgaccaccagaacccagctgccccccgcctacaccaacagcttcaccagaggcgtgtactaccccgacaaggtgttcagaagcagcgtgctgcacagcacccaggacctgttcctgcccttcttcagcaacgtgacctggttccacgtgatcagcggcaccaacggcaccaagagattcgacaaccccgtgctgcccttcaacgacggcgtgtacttcgccagcatcgagaagagcaacatcatcagaggctggatcttcggcaccaccctggacagcaagacccagagcctgctgatcgtgaacaacgccaccaacgtggtgatcaaggtgtgcgagttccagttctgcaacgaccccttcctggaccacaagaacaacaagagctggatggagagcgagttcagagtgtacagcagcgccaacaactgcaccttcgagtacgtgagccagcccttcctgatggacctggagggcaagcagggcaacttcaagaacctgagagagttcgtgttcaagaacatcgacggctacttcaagatctacagcaagcacacccccatcatcgtgagagagcccgaggacctgccccagggcttcagcgccctggagcccctggtggacctgcccatcggcatcaacatcaccagattccagaccctgctggccctgcacagaagctacctgacccccggcgacagcagcagcggctggaccgccggcgccgccgcctactacgtgggctacctgcagcccagaaccttcctgctgaagtacaacgagaacggcaccatcaccgacgccgtggactgcgccctggaccccctgagcgagaccaagtgcaccctgaagagcttcaccgtggagaagggcatctaccagaccagcaacttcagagtgcagcccaccgagagcatcgtgagattccccaacatcaccaacctgtgccccttcgacgaggtgttcaacgccaccagattcgccagcgtgtacgcctggaacagaaagagaatcagcaactgcgtggccgactacagcgtgctgtacaacctggcccccttcttcaccttcaagtgctacggcgtgagccccaccaagctgaacgacctgtgcttcaccaacgtgtacgccgacagcttcgtgatcagaggcgacgaggtgagacagatcgcccccggccagaccggcaacatcgccgactacaactacaagctgcccgacgacttcaccggctgcgtgatcgcctggaacagcaacaagctggacagcaaggtgagcggcaactacaactacctgtacagactgttcagaaagagcaacctgaagcccttcgagagagacatcagcaccgagatctaccaggccggcaacaagccctgcaacggcgtggccggcttcaactgctacttccccctgaagagctacagcttcagacccacctacggcgtgggccaccagccctacagagtggtggtgctgagcttcgagctgctgcacgcccccgccaccgtgtgcggccccaagaagagcaccaacctggtgaagaacaagtgcgtgaacttcaacttcaacggcctgaagggcaccggcgtgctgaccgagagcaacaagaagttcctgcccttccagcagttcggcagagacatcgccgacaccaccgacgccgtgagagacccccagaccctggagatcctggacatcaccccctgcagcttcggcggcgtgagcgtgatcacccccggcaccaacaccagcaaccaggtggccgtgctgtaccagggcgtgaactgcaccgaggtgcccgtggccatccacgccgaccagctgacccccacctggagagtgtacagcaccggcagcaacgtgttccagaccagagccggctgcctgatcggcgccgagtacgtgaacaacagctacgagtgcgacatccccatcggcgccggcatctgcgccagctaccagacccagaccaagagccaccagcaggcccagagcgtggccagccagagcatcatcgcctacaccatgagcctgggcgccgagaacagcgtggcctacagcaacaacagcatcgccatccccaccaacttcaccatcagcgtgaccaccgagatcctgcccgtgagcatgaccaagaccagcgtggactgcaccatgtacatctgcggcgacagcaccgagtgcagcaacctgctgctgcagtacggcagcttctgcacccagctgaagagagccctgaccggcatcgccgtggagcaggacaagaacacccaggaggtgttcgcccaggtgaagcagatctacaagaccccccccatcaagtacttcggcggcttcaacttcagccagatcctgcccgaccccagcaagcccagcaagagaagcttcatcgaggacctgctgttcaacaaggtgaccctggccgacgccggcttcatcaagcagtacggcgactgcctgggcgacatcgccgccagagacctgatctgcgcccagaagttcaagggcctgaccgtgctgccccccctgctgaccgacgagatgatcgcccagtacaccagcgccctgctggccggcaccatcaccagcggctggaccttcggcgccggcgccgccctgcagatccccttcgccatgcagatggcctacagattcaacggcatcggcgtgacccagaacgtgctgtacgagaaccagaagctgatcgccaaccagttcaacagcgccatcggcaagatccaggacagcctgagcagcaccgccagcgccctgggcaagctgcaggacgtggtgaaccacaacgcccaggccctgaacaccctggtgaagcagctgagcagcaagttcggcgccatcagcagcgtgctgaacgacatcttcagcagactggacccccccgaggccgaggtgcagatcgacagactgatcaccggcagactgcagagcctgcagacctacgtgacccagcagctgatcagagccgccgagatcagagccagcgccaacctggccgccaccaagatgagcgagtgcgtgctgggccagagcaagagagtggacttctgcggcaagggctaccacctgatgagcttcccccagagcgccccccacggcgtggtgttcctgcacgtgacctacgtgcccgcccaggagaagaacttcaccaccgcccccgccatctgccacgacggcaaggcccacttccccagagagggcgtgttcgtgagcaacggcacccactggttcgtgacccagagaaacttctacgagccccagatcatcaccaccgacaacaccttcgtgagcggcaactgcgacgtggtgatcggcatcgtgaacaacaccgtgtacgaccccctgcagcccgagctggacagcttcaaggaggagctggacaagtacttcaagaaccacaccagccccgacgtggacctgggcgacatcagcggcatcaacgccagcgtggtgaacatccagaaggagatcgacagactgaacgaggtggccaagaacctgaacgagagcctgatcgacctgcaggagctgggcaagtacgagcagtacatcaagtggccctggtacatctggctgggcttcatcgccggcctgatcgccatcgtgatggtgaccatcatgctgtgctgcatgaccagctgctgcagctgcctgaagggctgctgcagctgcggcagctgctgcaagttcgacgaggacgacagcgagcccgtgctgaagggcgtgaagctgcactacacctga

SEQ ID NO: 4 - protein, 1270 aa, synthetic construct
MFVFLVLLPLVSSQCVNLTTRTQLPPAYTNSFTRGVYYPDKVFRSSVLHSTQDLFLPFFSNVTWFHVISGTNGTKRFDNPVLPFNDGVYFASIEKSNIIRGWIFGTTLDSKTQSLLIVNNATNVVIKVCEFQFCNDPFLDHKNNKSWMESEFRVYSSANNCTFEYVSQPFLMDLEGKQGNFKNLREFVFKNIDGYFKIYSKHTPIIVREPEDLPQGFSALEPLVDLPIGINITRFQTLLALHRSYLTPGDSSSGWTAGAAAYYVGYLQPRTFLLKYNENGTITDAVDCALDPLSETKCTLKSFTVEKGIYQTSNFRVQPTESIVRFPNITNLCPFDEVFNATRFASVYAWNRKRISNCVADYSVLYNLAPFFTFKCYGVSPTKLNDLCFTNVYADSFVIRGDEVRQIAPGQTGNIADYNYKLPDDFTGCVIAWNSNKLDSKVSGNYNYLYRLFRKSNLKPFERDISTEIYQAGNKPCNGVAGFNCYFPLKSYSFRPTYGVGHQPYRVVVLSFELLHAPATVCGPKKSTNLVKNKCVNFNFNGLKGTGVLTESNKKFLPFQQFGRDIADTTDAVRDPQTLEILDITPCSFGGVSVITPGTNTSNQVAVLYQGVNCTEVPVAIHADQLTPTWRVYSTGSNVFQTRAGCLIGAEYVNNSYECDIPIGAGICASYQTQTKSHQQAQSVASQSIIAYTMSLGAENSVAYSNNSIAIPTNFTISVTTEILPVSMTKTSVDCTMYICGDSTECSNLLLQYGSFCTQLKRALTGIAVEQDKNTQEVFAQVKQIYKTPPIKYFGGFNFSQILPDPSKPSKRSFIEDLLFNKVTLADAGFIKQYGDCLGDIAARDLICAQKFKGLTVLPPLLTDEMIAQYTSALLAGTITSGWTFGAGAALQIPFAMQMAYRFNGIGVTQNVLYENQKLIANQFNSAIGKIQDSLSSTASALGKLQDVVNHNAQALNTLVKQLSSKFGAISSVLNDIFSRLDPPEAEVQIDRLITGRLQSLQTYVTQQLIRAAEIRASANLAATKMSECVLGQSKRVDFCGKGYHLMSFPQSAPHGVVFLHVTYVPAQEKNFTTAPAICHDGKAHFPREGVFVSNGTHWFVTQRNFYEPQIITTDNTFVSGNCDVVIGIVNNTVYDPLQPELDSFKEELDKYFKNHTSPDVDLGDISGINASVVNIQKEIDRLNEVAKNLNESLIDLQELGKYEQYIKWPWYIWLGFIAGLIAIVMVTIMLCCMTSCCSCLKGCCSCGSCCKFDEDDSEPVLKGVKLHYT